European Patent Application EP 4 527 926 A1, published March 26, 2025. Title: BAC ENGINEERING WITH HALF-SITE DIRECTED FRAGMENT REPLACEMENT. Applicant: Albert-Ludwigs-Universität Freiburg. Application EP. The sequence listing filed with the application follows.

SEQUENCE LISTING (27 sequences)

SEQ ID NO: 1 - DNA, 88 bp, synthetic construct
  source 1..88: mol_type = other DNA
tattggcttcaatccaaaataaggtatattattgatgatgcctccggggtccactgcaattacttctcgaccaattctcatgtttgac

SEQ ID NO: 2 - DNA, 86 bp, synthetic construct
  source 1..86: mol_type = other DNA
tattggcttcaatccaaaataaggtatattattgatgatgcctccggggtccactgcaattataaactcgacagcgacacacttgc

SEQ ID NO: 3 - DNA, 82 bp, synthetic construct
  source 1..82: mol_type = other DNA
tttgggtaacaggaggggggtgttcctaccttaccaatgcaatttaaattcgtgtgggcggacaataaagtcttaaactgaa

SEQ ID NO: 4 - DNA, 75 bp, synthetic construct
  source 1..75: mol_type = other DNA
gcaagacacttgcttgatccaaatccaaacagagtctggttttttatttaaattgtgggcggacaaaatagttgg

SEQ ID NO: 5 - DNA, 67 bp, synthetic construct
  source 1..67: mol_type = other DNA
gaataagaggaagtgaaatctgaataatttaaattcgtgtgggcggacaataaagtcttaaactgaa

SEQ ID NO: 6 - DNA, 59 bp, synthetic construct
  source 1..59: mol_type = other DNA
ttcccacccttaagccacgcccacacatttaaataaatgtgggcggacaaaatagttgg

SEQ ID NO: 7 - DNA, 40 bp, synthetic construct
  source 1..40: mol_type = other DNA
ccgcgtgtgtacctctacctggagtttttcccacggtgga

SEQ ID NO: 8 - DNA, 40 bp, synthetic construct
  source 1..40: mol_type = other DNA
tccaccgtgggaaaaactccaggtagaggtacacacgcgg

SEQ ID NO: 9 - DNA, 22 bp, synthetic construct
  source 1..22: mol_type = other DNA
gacgggtaaaacgacggccagt

SEQ ID NO: 10 - DNA, 30 bp, synthetic construct
  source 1..30: mol_type = other DNA
taatgactcagtacaggaaacagctatgac

SEQ ID NO: 11 - DNA, 38 bp, synthetic construct
  source 1..38: mol_type = other DNA
aatggaagagctcccatgtcagccgttaagtgttcctg

SEQ ID NO: 12 - DNA, 47 bp, synthetic construct
  source 1..47: mol_type = other DNA
cattgaagagcttagaaaaactcatcgagcatcaaatgaaactgcaa

SEQ ID NO: 13 - DNA, 82 bp, synthetic construct
  source 1..82: mol_type = other DNA
gctcgatgagtttttctaagctcttcaatggaataagaggaagtgaaatctgaataatttgacgggtaaaacgacggccagt

SEQ ID NO: 14 - DNA, 86 bp, synthetic construct
  source 1..86: mol_type = other DNA
cttaacggctgacatgggagctcttccattttcccacccttaagccacgcccacacatttcagtaccatagagcccaccgcatccc

SEQ ID NO: 15 - DNA, 27 bp, synthetic construct
  source 1..27: mol_type = other DNA
catgcaagcttggcgtaatcatggtca

SEQ ID NO: 16 - DNA, 20 bp, synthetic construct
  source 1..20: mol_type = other DNA
gatccccgggtaccgagctc

SEQ ID NO: 17 - DNA, 66 bp, synthetic construct
  source 1..66: mol_type = other DNA
cgtcaccgcatgtgagcagacttcctctgccctctccggaaaccgcattgggaggggaggaagcct

SEQ ID NO: 18 - DNA, 41 bp, synthetic construct
  source 1..41: mol_type = other DNA
ctaccttaccaatgcaatttgagtcacactaagatattgct

SEQ ID NO: 19 - DNA, 47 bp, synthetic construct
  source 1..47: mol_type = other DNA
cagagtctggttttttatttatgtttcagggcaaggcggagccggag

SEQ ID NO: 20 - DNA, 63 bp, synthetic construct
  source 1..63: mol_type = other DNA
tctgctcacatgcggtgacgtggaggagaatcccgggccagcccagtccaagcacggcctgac

SEQ ID NO: 21 - DNA, 66 bp, synthetic construct
  source 1..66: mol_type = other DNA
atatgttttatgtatccagtaaccattgtannnnatgactctagaggatccccgggtaccgagctc

SEQ ID NO: 22 - DNA, 64 bp, synthetic construct
  source 1..64: mol_type = other DNA
tacaatggttactggatacataaaacatatnnnntagtccatcggttgcccaaagtgttaagat

SEQ ID NO: 23 - DNA, 64 bp, synthetic construct
  source 1..64: mol_type = other DNA
attgcgggaaacggccctaggggtgatatannnnatcttaacactttgggcaaccgatggacta

SEQ ID NO: 24 - DNA, 66 bp, synthetic construct
  source 1..66: mol_type = other DNA
tacaatggttactggatacataaaacatatnnnntagacctgcaggcatgcaagcttggcgtaatc

SEQ ID NO: 25 - DNA, 66 bp, synthetic construct
  source 1..66: mol_type = other DNA
gattacgccaagcttgcatgcctgcaggtctannnnatcttaacactttgggcaaccgatggacta

SEQ ID NO: 26 - DNA, 66 bp, synthetic construct
  source 1..66: mol_type = other DNA
tatatcacccctagggccgtttcccgcaatnnnntagacctgcaggcatgcaagcttggcgtaatc

SEQ ID NO: 27 - DNA, 30 bp, synthetic construct
  source 1..30: mol_type = other DNA
gacctgcaggcatgcaagcttggcgtaatc